European Patent Application EP 4 226 944 A2, published August 16, 2023. Title: TUMOR MUTATIONAL LOAD. Applicant: MEMORIAL SLOAN KETTERING CANCER CENTER. The sequence listing filed with the application follows.

SEQUENCE LISTING (39 sequences)

SEQ ID NO: 1 - protein, 9 aa, Homo sapiens
TESPFEQHI

SEQ ID NO: 2 - protein, 4 aa, unidentified
  REGION 1..4: note = CTLA-4 sequence
YVKM

SEQ ID NO: 3 - protein, 9 aa, Homo sapiens
TKSPFEQHI

SEQ ID NO: 4 - protein, 9 aa, Homo sapiens
EEKLSVVLF

SEQ ID NO: 5 - protein, 11 aa, Homo sapiens
SELFRSRLDSY

SEQ ID NO: 6 - protein, 9 aa, Homo sapiens
KELEGILLP

SEQ ID NO: 7 - protein, 10 aa, Homo sapiens
MEVDPIGHLY

SEQ ID NO: 8 - protein, 9 aa, Homo sapiens
SEIWRDIDF

SEQ ID NO: 9 - protein, 9 aa, Homo sapiens
EEKLIVVLF

SEQ ID NO: 10 - protein, 11 aa, Homo sapiens
SELFRSGLDSY

SEQ ID NO: 11 - protein, 9 aa, Homo sapiens
KELEGILLL

SEQ ID NO: 12 - protein, 8 aa, synthetic construct
  REGION 1..8: note = Synthetic peptide
GGRKKYKL

SEQ ID NO: 13 - protein, 8 aa, synthetic construct
  REGION 1..8: note = Synthetic peptide
GGKKKYQL

SEQ ID NO: 14 - protein, 8 aa, synthetic construct
  REGION 1..8: note = Synthetic peptide
GGKKKYKL

SEQ ID NO: 15 - protein, 8 aa, synthetic construct
  REGION 1..8: note = Synthetic peptide
GGKKKYRL

SEQ ID NO: 16 - protein, 8 aa, synthetic construct
  REGION 1..8: note = Synthetic peptide
GGKKRYKL

SEQ ID NO: 17 - protein, 9 aa, synthetic construct
  REGION 1..9: note = Synthetic peptide
HSKKKCDEL

SEQ ID NO: 18 - protein, 8 aa, synthetic construct
  REGION 1..8: note = Synthetic peptide
HSKKKCDE

SEQ ID NO: 19 - protein, 7 aa, synthetic construct
  REGION 1..7: note = Synthetic peptide
ELKRKMI

SEQ ID NO: 20 - protein, 7 aa, synthetic construct
  REGION 1..7: note = Synthetic peptide
ELNRKMI

SEQ ID NO: 21 - protein, 7 aa, synthetic construct
  REGION 1..7: note = Synthetic peptide
ELRRKMM

SEQ ID NO: 22 - protein, 7 aa, synthetic construct
  REGION 1..7: note = Synthetic peptide
DELEIKA

SEQ ID NO: 23 - protein, 8 aa, synthetic construct
  REGION 1..8: note = Synthetic peptide
VPLRPMTY

SEQ ID NO: 24 - protein, 11 aa, unidentified
  source 1..11: note = Organism - Epstein Barr Virus
LPEPLPQGQLT

SEQ ID NO: 25 - protein, 9 aa, unidentified
  source 1..9: note = Organism - Epstein Barr Virus
EPLPQGQLT

SEQ ID NO: 26 - protein, 7 aa, synthetic construct
  REGION 1..7: note = Synthetic peptide
KPIVVLH

SEQ ID NO: 27 - protein, 11 aa, unidentified
  source 1..11: note = Organism - Epstein Barr Virus
EPLPQGQLTAY

SEQ ID NO: 28 - protein, 10 aa, synthetic construct
  REGION 1..10: note = Synthetic peptide
RPQVPLRPMT

SEQ ID NO: 29 - protein, 9 aa, synthetic construct
  REGION 1..9: note = Synthetic peptide
EEYLQAFTY

SEQ ID NO: 30 - protein, 9 aa, synthetic construct
  REGION 1..9: note = Synthetic peptide
EEYLKAWTF

SEQ ID NO: 31 - protein, 8 aa, synthetic construct
  REGION 1..8: note = Synthetic peptide
EEPTVIKK

SEQ ID NO: 32 - protein, 7 aa, synthetic construct
  REGION 1..7: note = Synthetic peptide
EEFGRAY

SEQ ID NO: 33 - protein, 5 aa, unidentified
  source 1..5: note = Organism - Human immunodeficiency virus
LPPVV

SEQ ID NO: 34 - protein, 9 aa, unidentified
  source 1..9: note = Organism - Plasmodium falciparum
KPIVQYDNF

SEQ ID NO: 35 - protein, 8 aa, synthetic construct
  REGION 1..8: note = Synthetic peptide
LSSPVTKS

SEQ ID NO: 36 - protein, 10 aa, synthetic construct
  REGION 1..10: note = Synthetic peptide
RVAQLENVYI

SEQ ID NO: 37 - protein, 10 aa, synthetic construct
  REGION 1..10: note = Synthetic peptide
LTTKLTNTNI

SEQ ID NO: 38 - protein, 9 aa, synthetic construct
  SITE 1: note = X can be any amino acid
  SITE 7..8: note = X can be any amino acid
  REGION 1..9: note = Synthetic peptide
  SITE 5: note = X can be any amino acid
XEIPXVXXY

SEQ ID NO: 39 - protein, 6 aa, unidentified
  source 1..6: note = Organism - Human immunodeficiency virus
TAFTIP